European Patent Specification EP 3 673 035 B1, published October 22, 2025. Title: Verbesserte Pflegeeigenschaften von Polyester Textilien II. Applicant: Henkel AG & Co. KGaA. The sequence listing filed with the application follows.

SEQUENCE LISTING (3 sequences)

SEQ ID NO: 1 - protein, 265 aa, isolated from leaf/branch compost
SPSVEAQSNPYQRGPNPTRSALTADGPFSVATYTVSRLSVSGFGGGVIYYPTGTSLTFGGIAMSPGYTADASSLAWLGRRLASHGFVVLVINTNSRFDYPDSRASQLSAALNYLRTSSPSAVRARLDANRLAVAGHSMGGGGTLRIAEQNPSLKAAVPLTPWHTDKTFNTSVPVLIVGAEADTVAPVSQHAIPFYQNLPSTTPKVYVELDNASHFAPNSNNAAISVYTISWMKLWVDNDTRYRQFLCNVNDPALSDFRTNNRHCQ

SEQ ID NO: 2 - protein, 293 aa, isolated from leaf/branch compost
MDGVLWRVRTAALMAALLALAAWALVWASPSVEAQSNPYQRGPNPTRSALTADGPFSVATYTVSRLSVSGFGGGVIYYPTGTSLTFGGIAMSPGYTADASSLAWLGRRLASHGFVVLVINTNSRFDYPDSRASQLSAALNYLRTSSPSAVRARLDANRLAVAGHSMGGGGTLRIAEQNPSLKAAVPLTPWHTDKTFNTSVPVLIVGAEADTVAPVSQHAIPFYQNLPSTTPKVYVELDNASHFAPNSNNAAISVYTISWMKLWVDNDTRYRQFLCNVNDPALSDFRTNNRHCQ

SEQ ID NO: 3 - DNA, 798 bp, Artificial
  Coding sequence for LC cutinase, codon-optimized for E.coli expression
atgagcccgagcgttgaagcacagagcaatccgtatcagcgtggtccgaatccgacccgtagcgcactgaccgcagatggtccgtttagcgttgcaacctataccgttagccgtctgagcgttagcggttttggtggtggtgttatctattatccgaccggcaccagcctgacctttggtggtattgcaatgagtccgggttatacagcagatgcaagcagcctggcatggctgggtcgtcgtctggcaagccatggttttgttgttctggtgattaataccaacagccgctttgattatccggattcacgtgcaagccagctgagcgcagcactgaattatctgcgtaccagcagcccgagtgcagttcgtgcacgtctggatgcaaatcgtctggccgttgcaggtcatagcatgggtggcggtggcaccctgcgtattgcagaacagaatccgagcctgaaagcagcagttccgctgaccccgtggcataccgataaaacctttaataccagcgttccggttctgattgttggtgcagaagcagataccgttgcaccggttagccagcatgcaattccgttttatcagaatctgccgagcaccaccccgaaagtttatgttgaactggataatgcaagccactttgcaccgaatagcaataatgcagcaattagcgtttataccatcagctggatgaaactgtgggttgataatgatacccgttatcgtcagtttctgtgcaatgttaatgatccggcactgagcgattttcgtaccaataatcgtcattgtcag